European Patent Application EP 4 520 819 A1, published March 12, 2025. Title: 一种用于合成麦角硫因的化学-酶偶联方法. Applicant: 中国科学院上海有机化学研究所. Application WO. The sequence listing filed with the application follows.

SEQUENCE LISTING (62 sequences)

SEQ ID NO: 1 - protein, 773 aa, synthetic construct
  REGION 1..773: note = SPEGT1
MTEIENIGALEVLFSPESIEQSLKRCQLPSTLLYDEKGLRLFDEITNLKEYYLYESELDILKKFSDSIANQLLSPDLPNTVIELGCGNMRKTKLLLDAFEKKGCDVHFYALDLNEAELQKGLQELRQTTNYQHVKVSGICGCFERLLQCLDRFRSEPNSRISMLYLGASIGNFDRKSAASFLRSFASRLNIHDNLLISFDHRNKAELVQLAYDDPYRITEKFEKNILASVNAVFGENLFDENDWEYKSVYDEDLGVHRAYLQAKNEVTVIKGPMFFQFKPSHLILIEESWKNSDQECRQIIEKGDFKLVSKYESTIADYSTYVITKQFPAMLQLPLQPCPSLAEWDALRKVWLFITNKLLNKDNMYTAWIPLRHPPIFYIGHVPVFNDIYLTKIVKNKATANKKHFWEWFQRGIDPDIEDPSKCHWHSEVPESWPSPDQLREYEKESWEYHIVKLCKAMDELSTSEKRILWLCYEHVAMHVETTLYIYVQSFQNANQTVSICGSLPEPAEKLTKAPLWVNVPETEIAVGMPLTTQYTSVGSNLQSSDLSAHENTDELFYFAWDNEKPMRKKLVSSFSIANRPISNGEYLDFINKKSKTERVYPKQWAEIDGTLYIRTMYGLLPLDDYLGWPVMTSYDDLNNYASSQGCRLPTEDELNCFYDRVLERTDEPYVSTEGKATGFQQLHPLALSDNSSNQIFTGAWEWTSTVLEKHEDFEPEELYPDYTRDFFDGKHNVVLGGSFATATRISNRRSFRNFYQAGYKYAWIGARLVKN

SEQ ID NO: 2 - DNA, 2322 bp, synthetic construct
  misc_feature 1..2322: note = spegt1
  source 1..2322: mol_type = other DNA
atgaccgaaattgagaacatcggtgccctggaagtgctgttttctccggaaagtattgaacagagtctgaaacgttgccagctgccgagtaccctgctgtatgatgagaaaggtctgcgcctgtttgatgaaatcaccaatctgaaagaatactacctgtatgaaagcgaactggatattctgaagaaattcagcgatagcattgccaatcagctgctgagtccggatctgccgaataccgttattgaactgggctgtggcaatatgcgtaagactaaactgctgctggatgcctttgagaagaaaggctgcgatgttcatttctatgccctggatctgaatgaagccgaactgcagaaaggtctgcaggaactgcgccagaccaccaactatcagcatgttaaagtgagtggtatttgcggttgtttcgaacgcctgctgcagtgtctggatcgtttccgtagcgaaccgaatagtcgtattagcatgctgtatctgggtgcaagtattggtaacttcgatcgcaaatcagccgcaagtttcctgcgtagtttcgcaagccgtctgaacatccatgataatctgctgattagtttcgatcatcgcaacaaagccgaactggttcagctggcctatgatgatccgtatcgcattaccgagaaattcgagaagaacattctggccagcgttaatgcagtgtttggcgagaatctgtttgatgagaatgattgggaatacaaatccgtttatgacgaagatctgggtgtgcatcgcgcatatctgcaggcaaagaatgaagttaccgtgatcaaaggtccgatgttctttcagttcaaaccgagtcatctgattctgattgaagaaagttggaagaatagtgatcaggaatgccgtcagatcatcgagaaaggcgatttcaaactggttagcaaatacgaaagtaccattgccgattacagcacctatgtgattaccaaacagtttccagccatgctgcagctgccgctgcagccttgtccgagcctggcagaatgggatgccctgcgcaaagtgtggctgttcattaccaacaaactgctgaataaggacaatatgtacaccgcctggattccgctgcgtcatccaccgatcttctacattggccatgtgccggtgttcaacgatatctacctgaccaagattgtgaagaataaggcaaccgccaataagaaacatttctgggaatggtttcagcgtggtattgatccggatattgaagatccgagcaaatgccattggcatagtgaagttccggaaagttggccgtctccggatcagctgcgtgaatatgagaaagaaagttgggaatatcatatcgtgaaactgtgtaaagcaatggatgaactgagtaccagtgagaaacgtattctgtggctgtgttatgaacatgttgccatgcatgtggaaaccaccctgtacatctatgtgcagagctttcagaatgcaaatcagaccgttagcatttgtggcagtctgccagaaccggcagagaaactgaccaaagcacctctgtgggtgaatgtgccggaaaccgaaattgcagttggcatgccgctgaccacccagtataccagtgtgggtagcaatctgcagagcagtgatctgagcgcacatgagaataccgatgaactgttctatttcgcatgggataatgagaaaccgatgcgtaagaaactggtgagcagctttagtattgccaatcgtccgattagtaatggtgaatatctggatttcatcaataagaaatccaagaccgaacgtgtttatccgaaacagtgggcagaaattgatggtaccctgtatatccgtaccatgtatggcctgctgccgctggatgattatctgggctggccagttatgaccagttatgatgatctgaacaattacgcaagtagccagggctgccgtctgccgaccgaagatgaactgaattgtttctatgatcgtgttctggaacgcaccgatgaaccgtatgtgagtaccgaaggcaaagccaccggctttcagcagctgcatccgctggcactgagcgataacagcagtaatcagatctttaccggtgcctgggaatggaccagtaccgttctggagaaacatgaagatttcgaaccggaagaactgtatccggattacacccgtgatttctttgatggcaaacataatgtggtgctgggtggtagctttgccaccgcaacccgtattagtaatcgtcgtagtttccgtaacttctaccaagccggttacaaatacgcctggattggtgcacgtctggtgaaaaactaa

SEQ ID NO: 3 - protein, 389 aa, synthetic construct
  REGION 1..389: note = SPEGT2
MAENNVYGHEMKKHFMLDPDYVNVNNGSCGTESLAVYNKHVQLLKEAQSKPDFMCNAYMPMYMEATRNEVAKLIGADSSNIVFCNSATDGISTVLLTFPWEQNDEILMLNVAYPTCTYAADFAKNQHNLRLDVIDVGVEIDEDLFLKEVEQRFLQSKPRAFICDILSSMPVILFPWEKVVKLCKKYNIVSIIDGAHAIGHIPMNLANVDPDFLFTNAHKWLNSPAACTVLYVSAKNHNLIEALPLSYGYGLREKESIAVDTLTNRFVNSFKQDLPKFIAVGEAIKFRKSIGGEEKIQQYCHEIALKGAEIISKELGTSFIKPPYPVAMVNVEVPLRNIPSIETQKVFWPKYNTFLRFMEFKGKFYTRLSGAVYLEESDFYYIAKVIKDF

SEQ ID NO: 4 - DNA, 1179 bp, synthetic construct
  misc_feature 1..1179: note = SPEGT2
  source 1..1179: mol_type = other DNA
atggctgagaacaacgtgtacggccacgaaatgaaaaaacatttcatgctggatcctgactatgtaaacgtgaacaacggtagctgcggtaccgaatccctggctgtttacaacaaacacgttcagctgctgaaagaagctcagtccaaaccggacttcatgtgtaacgcttacatgccgatgtacatggaagcgacccgtaatgaagtcgccaaactgatcggtgcggactcttccaacatcgtgttctgcaacagcgcaacggacggcatttctactgtcctgctgaccttcccgtgggagcagaacgatgaaatcctgatgctgaacgttgcgtatccgacctgtacctacgctgcggactttgcgaaaaaccagcataacctgcgcctggacgttatcgatgttggtgttgaaatcgatgaagatctgtttctgaaagaagttgaacagcgcttcctgcagtccaaaccgcgtgcgttcatctgcgacatcctgtcctctatgccggtcattctgtttccgtgggagaaagtggtgaagctgtgcaaaaaatacaatattgtgtccatcatcgacggtgcgcacgcgattggccacatcccgatgaatctggctaacgtggatccggattttctgttcaccaacgcgcacaaatggctgaactctccggcagcgtgcaccgtgctgtacgtttctgcaaagaaccacaacctgatcgaagcactgccactgagctacggctacggcctgcgtgaaaaagaatctattgcagttgacaccctgaccaaccgcttcgttaacagcttcaaacaagatctgccgaaattcatcgcagtcggcgaagctatcaaattccgtaagagcatcggtggcgaagaaaaaatccagcagtactgtcacgaaatcgcgctgaaaggtgcggagattatctctaaagagctgggcacctccttcatcaaaccgccgtatccagttgccatggttaacgttgaggttccgctgcgtaacattccaagcatcgaaacccagaaagttttctggccgaaatataataccttcctgcgtttcatggaattcaaaggcaaattctacacccgtctgtctggcgccgtgtatctggaagaatctgacttctactatatcgccaaagtaatcaaggacttctgttccctgtaa

SEQ ID NO: 5 - protein, 445 aa, synthetic construct
  REGION 1..445: note = SPEGT1-tr
PAMLQLPLQPCPSLAEWDALRKVWLFITNKLLNKDNMYTAWIPLRHPPIFYIGHVPVFNDIYLTKIVKNKATANKKHFWEWFQRGIDPDIEDPSKCHWHSEVPESWPSPDQLREYEKESWEYHIVKLCKAMDELSTSEKRILWLCYEHVAMHVETTLYIYVQSFQNANQTVSICGSLPEPAEKLTKAPLWVNVPETEIAVGMPLTTQYTSVGSNLQSSDLSAHENTDELFYFAWDNEKPMRKKLVSSFSIANRPISNGEYLDFINKKSKTERVYPKQWAEIDGTLYIRTMYGLLPLDDYLGWPVMTSYDDLNNYASSQGCRLPTEDELNCFYDRVLERTDEPYVSTEGKATGFQQLHPLALSDNSSNQIFTGAWEWTSTVLEKHEDFEPEELYPDYTRDFFDGKHNVVLGGSFATATRISNRRSFRNFYQAGYKYAWIGARLVKN

SEQ ID NO: 6 - DNA, 1338 bp, synthetic construct
  misc_feature 1..1338: note = spegt1-tr
  source 1..1338: mol_type = other DNA
ccagccatgctgcagctgccgctgcagccttgtccgagcctggcagaatgggatgccctgcgcaaagtgtggctgttcattaccaacaaactgctgaataaggacaatatgtacaccgcctggattccgctgcgtcatccaccgatcttctacattggccatgtgccggtgttcaacgatatctacctgaccaagattgtgaagaataaggcaaccgccaataagaaacatttctgggaatggtttcagcgtggtattgatccggatattgaagatccgagcaaatgccattggcatagtgaagttccggaaagttggccgtctccggatcagctgcgtgaatatgagaaagaaagttgggaatatcatatcgtgaaactgtgtaaagcaatggatgaactgagtaccagtgagaaacgtattctgtggctgtgttatgaacatgttgccatgcatgtggaaaccaccctgtacatctatgtgcagagctttcagaatgcaaatcagaccgttagcatttgtggcagtctgccagaaccggcagagaaactgaccaaagcacctctgtgggtgaatgtgccggaaaccgaaattgcagttggcatgccgctgaccacccagtataccagtgtgggtagcaatctgcagagcagtgatctgagcgcacatgagaataccgatgaactgttctatttcgcatgggataatgagaaaccgatgcgtaagaaactggtgagcagctttagtattgccaatcgtccgattagtaatggtgaatatctggatttcatcaataagaaatccaagaccgaacgtgtttatccgaaacagtgggcagaaattgatggtaccctgtatatccgtaccatgtatggcctgctgccgctggatgattatctgggctggccagttatgaccagttatgatgatctgaacaattacgcaagtagccagggctgccgtctgccgaccgaagatgaactgaattgtttctatgatcgtgttctggaacgcaccgatgaaccgtatgtgagtaccgaaggcaaagccaccggctttcagcagctgcatccgctggcactgagcgataacagcagtaatcagatctttaccggtgcctgggaatggaccagtaccgttctggagaaacatgaagatttcgaaccggaagaactgtatccggattacacccgtgatttctttgatggcaaacataatgtggtgctgggtggtagctttgccaccgcaacccgtattagtaatcgtcgtagtttccgtaacttctaccaagccggttacaaatacgcctggattggtgcacgtctggtgaaaaactaa

SEQ ID NO: 7 - protein, 445 aa, synthetic construct
  REGION 1..445: note = SPEGT1-tr M10
PAMLQLPLQPCPSLAEWDALRKVWLFITNKLLNKDNMYTAWIPLRHPPILFIGHVPVFNDIYLTKIVKNKATANKKHFWEWFQRGIDPDIEDPSKCNWNSEVPESWPSPDQLREYEKESWEYHIVKLCKAMDELSTSEKRILWLCYEHVALHVETTLYIYVQSFQNANQTVSICGSLPEPAEKLTKAPLWVNVPETEIAVGMPLTTQYTSVGSNLQSSDLSAHENTDELFYFAWDNEKPMRKKLVSSFSIANRPISNGEYLDFINKKSKTERVYPKQWAEIDGTLYIRTMYGLLPLDDYLGWPVMTSYDDLNNYASSQGCRLPTEDELNCFYDRVLERTDEPYVSTEGKATGFQQLHPLALSDNSSNQIFTGAWECTSTVLEKHEDFEPEELYPDYTRDFFDGKLNVVLGGSFATATRISNRRSLRNFYQAGYKSAWIGARLVKN

SEQ ID NO: 8 - DNA, 1338 bp, synthetic construct
  misc_feature 1..1338: note = SPEGT1-tr M10
  source 1..1338: mol_type = other DNA
ccagccatgctgcagctgccgctgcagccttgtccgagcctggcagaatgggatgccctgcgcaaagtgtggctgttcattaccaacaaactgctgaataaggacaatatgtacaccgcctggattccgctgcgtcatccaccgatcctcttcattggccatgtgccggtattcaacgatatctacctgaccaagattgtgaagaataaggcaaccgccaataagaaacatttctgggaatggtttcagcgtggtattgatccggatattgaagatccgagcaaatgcaattggaacagtgaagttccggaaagttggccgtctccggatcagctgcgtgaatatgagaaagaaagttgggaatatcatatcgtgaagctgtgtaaagcaatggatgaactgagtaccagtgagaaacgtattctgtggctgtgttatgaacatgttgccctgcatgtggaaaccaccctgtacatctatgtgcagagctttcagaatgcaaatcagaccgttagcatttgtggcagtctgccagaaccggcagagaaactgaccaaagcacctctgtgggtgaatgtgccggaaaccgaaattgcagttggcatgccgctgaccacccagtataccagtgtgggtagcaatctgcagagcagtgatctgagcgcacatgagaataccgatgaactgttctatttcgcatgggataatgagaaaccgatgcgtaagaaactggtgagcagctttagtattgccaatcgtccgattagtaatggtgaatatctggatttcatcaataagaaatccaagaccgaacgtgtttatccgaaacagtgggcagaaattgatggtaccctgtatatccgtaccatgtatggcctgctgccgctggatgattatctgggctggccagttatgaccagttatgatgatctgaacaattacgcaagtagccagggctgccgtctgccgaccgaagatgaactgaattgtttctatgatcgtgttctggaacgcaccgatgaaccgtatgtgagtaccgaaggcaaagccaccggctttcagcagctgcatccgctggcactgagcgataacagcagtaatcagatctttaccggtgcctgggaatgtaccagtaccgttctggagaaacatgaagatttcgaaccggaagaactgtacccggattacacccgtgatttctttgatggcaaacttaatgtggtgctgggtggtagctttgccaccgcaacccgtattagtaatcgtcgtagtctccgtaacttctaccaagccggttacaaatccgcctggattggtgcacgtctggtgaaaaactaa

SEQ ID NO: 9 - protein, 392 aa, synthetic construct
  REGION 1..392: note = SPEGT2 M3
MAENNVYGHEMKKHFMLDPDYVNVNNGPCGTESLAVYNKHVQLLKEAQSKPDFMCNAYMPMYMEATRNEVAKLIGADSSNIVFCNSATDGISTVLLTFPWEQNDEILMLNVAFPTCTYAADFAKNQHNLRLDVIDVGVEIDEDLFLKEVEQRFLQSKPRAFICDILASMPVILFPWEKVVKLCKKYNIVSIIDGAHAIGHIPMNLANVDPDFLFTNAHKWLNSPAACTVLYVSAKNHNLIEALPLSYGYGLREKESIAVDTLTNRFVNSFKQDLPKFIAVGEAIKFRKSIGGEEKIQQYCHEIALKGAEIISKELGTSFIKPPYPVAMVNVEVPLRNIPSIETQKVFWPKYNTFLRFMEFKGKFYTRLSGAVYLEESDFYYIAKVIKDFCSL

SEQ ID NO: 10 - DNA, 1179 bp, synthetic construct
  misc_feature 1..1179: note = SPEGT2 M3
  source 1..1179: mol_type = other DNA
atggctgagaacaacgtgtacggccacgaaatgaaaaaacatttcatgctggatcctgactatgtaaacgtgaacaacggtccctgcggtaccgaatccctggctgtttacaacaaacacgttcagctgctgaaagaagctcagtccaaaccggacttcatgtgtaacgcttacatgccgatgtacatggaagcgacccgtaatgaagtcgccaaactgatcggtgcggactcttccaacatcgtgttctgcaacagcgcaacggacggcatttctactgtcctgctgaccttcccgtgggagcagaacgatgaaatcctgatgctgaacgttgcgtttccgacctgtacctacgctgcggactttgcgaaaaaccagcataacctgcgcctggacgttatcgatgttggtgttgaaatcgatgaagatctgtttctgaaagaagttgaacagcgcttcctgcagtccaaaccgcgtgcgttcatctgcgacatcctggcctctatgccggtcattctgtttccgtgggagaaagtggtgaagctgtgcaaaaaatacaatattgtgtccatcatcgacggtgcgcacgcgattggccacatcccgatgaatctggctaacgtggatccggattttctgttcaccaacgcgcacaaatggctgaactctccggcagcgtgcaccgtgctgtacgtttctgcaaagaaccacaacctgatcgaagcactgccactgagctacggctacggcctgcgtgaaaaagaatctattgcagttgacaccctgaccaaccgcttcgttaacagcttcaaacaagatctgccgaaattcatcgcagtcggcgaagctatcaaattccgtaagagcatcggtggcgaagaaaaaatccagcagtactgtcacgaaatcgcgctgaaaggtgcggagattatctctaaagagctgggcacctccttcatcaaaccgccgtatccagttgccatggttaacgttgaggttccgctgcgtaacattccaagcatcgaaacccagaaagttttctggccgaaatataataccttcctgcgtttcatggaattcaaaggcaaattctacacccgtctgtctggcgccgtgtatctggaagaatctgacttctactatatcgccaaagtaatcaaggacttctgttccctgtaa

SEQ ID NO: 11 - protein, 437 aa, Schizosaccharomyces octosporus yFS286
PILPQIPKEASISLEEWSQTRDIWLFVTNKLLNDSNIFNVWIPLRHPFIFYMGHIPVFNDIYLSRIFENPATASKREYWDWFQRGIDPDVENPEQCHWHSQTPPKWPSPNELRSYEVASWQNHILKLLDGSHALSPSQKRILWLCYEHVAMHIETTLYIYVQSFQHPKQNNTLCGLPPSKNLKLKKDPSWIKFPNAQVLQGLPIRSDQKTKLNSEEPDEQEFFGWDNEKPLRMKQIPSFQIANRPISNGEYLDYLESKPADDKHYPKSWKVIDGKLYVTTMYGLLPLESYHSWPVMASFEELNDYAASKGCRLPTEEELNHFYDHVLHRKSETYVSTKGMATGFQQLHPANLKDDGTHQIFTGAWEWSSTVLDKHEGFEPEALYPDYTKDFFDGKHNVVLGGSFATVPRIANRRSFRNFYQRQYQYAWITARLAKSI

SEQ ID NO: 12 - DNA, 1311 bp, Schizosaccharomyces octosporus yFS286
  source 1..1311: mol_type = genomic DNA
ccgattctgccgcagattccgaaagaagcgagcattagcctggaagaatggagccagacccgcgatatttggctgtttgtgaccaacaaactgctgaacgatagcaacatttttaacgtgtggattccgctgcgccatccgtttattttttatatgggccatattccggtgtttaacgatatttatctgagccgcatttttgaaaacccggcgaccgcgagcaaacgcgaatattgggattggtttcagcgcggcattgatccggatgtggaaaacccggaacagtgccattggcatagccagaccccgccgaaatggccgagcccgaacgaactgcgcagctatgaagtggcgagctggcagaaccatattctgaaactgctggatggcagccatgcgctgagcccgagccagaaacgcattctgtggctgtgctatgaacatgtggcgatgcatattgaaaccaccctgtatatttatgtgcagagctttcagcatccgaaacagaacaacaccctgtgcggcctgccgccgagcaaaaacctgaaactgaaaaaagatccgagctggattaaatttccgaacgcgcaggtgctgcagggcctgccgattcgcagcgatcagaaaaccaaactgaacagcgaagaaccggatgaacaggaattttttggctgggataacgaaaaaccgctgcgcatgaaacagattccgagctttcagattgcgaaccgcccgattagcaacggcgaatatctggattatctggaaagcaaaccggcggatgataaacattatccgaaaagctggaaagtgattgatggcaaactgtatgtgaccaccatgtatggcctgctgccgctggaaagctatcatagctggccggtgatggcgagctttgaagaactgaacgattatgcggcgagcaaaggctgccgcctgccgaccgaagaagaactgaaccatttttatgatcatgtgctgcatcgcaaaagcgaaacctatgtgagcaccaaaggcatggcgaccggctttcagcagctgcatccggcgaacctgaaagatgatggcacccatcagatttttaccggcgcgtgggaatggagcagcaccgtgctggataaacatgaaggctttgaaccggaagcgctgtatccggattataccaaagatttttttgatggcaaacataacgtggtgctgggcggcagctttgcgaccgtgccgcgcattgcgaaccgccgcagctttcgcaacttttatcagcgccagtatcagtatgcgtggattaccgcgcgcctggcgaaaagcatt

SEQ ID NO: 13 - protein, 437 aa, Schizosaccharomyces cryophilus OY26
PKLPQLPKEAPISLREWSGIRDIWIFITNKLLNDSNIFKVWIPLRHPFVFYMGHIPVFNDIYLSRIFENPVTASKRQYWDWFQRGIDPDVENPENCHWHSQIPTNWPSPNELRSYEIASWQNHILKLYDGSHTLSPFQKRIVWLCYEHVAMHIETTLYIYVQSFQDPKQNNFICGLPPCKIPKLKKDPSWIKYYNGQVLLGLPVRNDRYSNSNPEEPDEQKFFGWDNEKPSRTNHVPSFQIANRPISNGEYLNFVNNKPEGDRRYPKLWKLIDGKLYLKTMYGLLPLDNYLSWPVMASFDELNAYAAFKGCRLPTEEELNYYYDQVLHRKSEAYVSTEGMATGFQQLHPAKLKDDETPQIFTGAWEWTSTVLEKHEGFEPEALYPDYTKDFFDGKHNVVLGGSFATVPRIANRRSFRNFYQRQYEYAWITARLAKGI

SEQ ID NO: 14 - DNA, 1311 bp, Schizosaccharomyces cryophilus OY26
  source 1..1311: mol_type = genomic DNA
ccgaaactgccacaactgccgaaagaagcaccaatcagcctgcgcgagtggagcggcatccgtgatatctggatcttcatcaccaacaaactgctgaacgatagcaacatcttcaaagtctggatccctctgcgccatccgttcgttttctatatgggtcacatcccggtatttaacgacatctacctgtctcgcatcttcgagaacccggtgactgcgtctaaacgtcagtactgggattggtttcagcgtggtattgatccggatgttgaaaatccggaaaactgccactggcactctcagatcccgactaactggccgagcccgaacgaactgcgttcctatgaaatcgcatcttggcagaaccacatcctgaaactgtatgatggtagccacaccctgtccccatttcagaagcgtatcgtatggctgtgctacgagcacgtggcaatgcacatcgaaactacgctgtacatttacgtgcagagcttccaggatccaaagcagaacaacttcatctgtggcctgccgccgtgcaaaatcccaaaactgaaaaaagacccgagctggattaaatactacaacggtcaggttctgctgggcctgccggtacgtaatgaccgttactctaactccaaccctgaagaaccggacgaacagaagttcttcggctgggataacgaaaagccgtctcgtaccaaccacgttccgtcttttcagattgcgaaccgtccgatttctaacggtgagtatctgaactttgtgaacaacaaaccggaaggcgatcgtcgttacccgaaactgtggaaactgatcgacggtaaactgtacctgaaaaccatgtacggcctgctgccgctggacaactacctgagctggccagttatggcttctttcgacgaactgaatgcgtacgcagcgtttaaaggctgtcgtctgccaaccgaagaagaactgaactactactacgaccaggttctgcatcgtaaatccgaagcatacgtttccaccgaaggtatggccactggtttccagcagctgcatccggccaaactgaaagatgatgaaactccgcagatttttacgggtgcttgggaatggaccagcactgttctggagaaacacgaaggtttcgaacctgaagcgctgtatccagactataccaaagactttttcgacggcaaacacaacgtggttctgggcggttctttcgctaccgttcctcgcattgctaatcgtcgcagcttccgtaatttctatcagcgccagtacgaatatgcgtggattacggcccgtctggccaagggtatc

SEQ ID NO: 15 - protein, 437 aa, Schizosaccharomyces osmophilus
PNLPQVPNEAPISLEEWSQTRAIWLFVTNKLLNDSNIFNVWIPLRHPFVFYMGHIPVFNDIYLSRIFENPATAPKREYWDWFQRGIDPDVENPEHCHWHSQAPPNWPSPNELRSYEVASWQNHILKLFDGSHALSPSQKRIVWLCYEHVAMHIETTLYIYVQSFQHPKQNNVICGLPPCKTPKLEKDPSWIKFSNGQVLLGLPIQNDRNTSSNPEKPDEQEFFGWDNEKPSRIEQVSPFQIANRPISNGEYLDYLESKPASDKHYPKLWKLIDGKLYLKTMYGLLPLENYSSWPVMASFEELNAYAASKGCRLPTEEELNYFYDHVLQRKSEAYVSTRGLATGFQQLHPAKLKDDGTPQIFTGAWEWSSTVLDKHEGFEPEALYPDYTQDFFDGKHNVVLGGSFATVPRIANRRSFRNFYQRQYQYAWITARLAKSI

SEQ ID NO: 16 - DNA, 1311 bp, Schizosaccharomyces osmophilus
  source 1..1311: mol_type = genomic DNA
ccgaacctgccgcaggtgccgaacgaagcgccgattagcctggaagaatggagccagacccgcgcgatttggctgtttgtgaccaacaaactgctgaacgatagcaacatttttaacgtgtggattccgctgcgccatccgtttgtgttttatatgggccatattccggtgtttaacgatatttatctgagccgcatttttgaaaacccggcgaccgcgccgaaacgcgaatattgggattggtttcagcgcggcattgatccggatgtggaaaacccggaacattgccattggcatagccaggcgccgccgaactggccgagcccgaacgaactgcgcagctatgaagtggcgagctggcagaaccatattctgaaactgtttgatggcagccatgcgctgagcccgagccagaaacgcattgtgtggctgtgctatgaacatgtggcgatgcatattgaaaccaccctgtatatttatgtgcagagctttcagcatccgaaacagaacaacgtgatttgcggcctgccgccgtgcaaaaccccgaaactggaaaaagatccgagctggattaaatttagcaacggccaggtgctgctgggcctgccgattcagaacgatcgcaacaccagcagcaacccggaaaaaccggatgaacaggaattttttggctgggataacgaaaaaccgagccgcattgaacaggtgagcccgtttcagattgcgaaccgcccgattagcaacggcgaatatctggattatctggaaagcaaaccggcgagcgataaacattatccgaaactgtggaaactgattgatggcaaactgtatctgaaaaccatgtatggcctgctgccgctggaaaactatagcagctggccggtgatggcgagctttgaagaactgaacgcgtatgcggcgagcaaaggctgccgcctgccgaccgaagaagaactgaactatttttatgatcatgtgctgcagcgcaaaagcgaagcgtatgtgagcacccgcggcctggcgaccggctttcagcagctgcatccggcgaaactgaaagatgatggcaccccgcagatttttaccggcgcgtgggaatggagcagcaccgtgctggataaacatgaaggctttgaaccggaagcgctgtatccggattatacccaggatttttttgatggcaaacataacgtggtgctgggcggcagctttgcgaccgtgccgcgcattgcgaaccgccgcagctttcgcaacttttatcagcgccagtatcagtatgcgtggattaccgcgcgcctggcgaaaagcatt

SEQ ID NO: 17 - protein, 431 aa, Schizosaccharomyces japonicus yFS275
FDVSRNPETPCPTLEEWTQIRLAWLYLVFKLYPRDLYFTELIPVRHPFIFYIGHVPAFNDIYLARLTDGKPTLGRKDYWDWFQRGIDPDLDNTKKCHWHSQPPEKWPSVEEVNEYERNVWSRLVSIYKQGEMSANMQRAMWMIYEHTAMHLETSYYILLQSDYHIISPNNFPPPIAPALQTDPTWVRVPESFITMGIPTTADGKETFYYGWDNEKPERQVSVRCFEIANRPISNGEYLSFLKETTQSKEEFEAAIPKTWLLKDEMLFAKSMYGPLPIEHVLGWPVATSYDELKQYANAKGCRLPTDYELRAFYDHVLKPNEETYVDTAGYATAFQQWYPKSLQDEEKPQIYTGLWEWTSTVLKEDLDFTPEELYPDYTRDFFDGKHNVVMGGSFTTVARIANRRSFRNFYQRKYPYAWIGARLVKVTNTLS

SEQ ID NO: 18 - DNA, 1293 bp, Schizosaccharomyces japonicus yFS275
  source 1..1293: mol_type = genomic DNA
tttgatgtgagccgtaacccggaaaccccgtgcccgaccctggaagaatggacccagattcgcctggcgtggctgtatctggtgtttaaactgtatccgcgcgatctgtattttaccgaactgattccggtgcgccatccgtttattttttatattggccatgtgccggcgtttaacgatatttatctggcgcgcctgaccgatggcaaaccgaccctgggccgcaaagattattgggattggtttcagcgcggcattgatccggatctggataacaccaaaaaatgccattggcatagccagccgccggaaaaatggccgagcgtggaagaagtgaacgaatatgaacgcaacgtgtggagccgcctggtgagcatttataaacagggcgaaatgagcgcgaacatgcagcgcgcgatgtggatgatttatgaacataccgcgatgcatctggaaaccagctattatattctgctgcagagcgattatcatattattagcccgaacaactttccgccgccgattgcgccggcgctgcagaccgatccgacctgggtgcgcgtgccggaaagctttattaccatgggcattccgaccaccgcggatggcaaagaaaccttttattatggctgggataacgaaaaaccggaacgccaggtgagcgtgcgctgctttgaaattgcgaaccgcccgattagcaacggcgaatatctgagctttctgaaagaaaccacccagagcaaagaagaatttgaagcggcgattccgaaaacctggctgctgaaagatgaaatgctgtttgcgaaaagcatgtatggcccgctgccgattgaacatgtgctgggctggccggtggcgaccagctatgatgaactgaaacagtatgcgaacgcgaaaggctgccgcctgccgaccgattatgaactgcgcgcgttttatgatcatgtgctgaaaccgaacgaagaaacctatgtggataccgcgggctatgcgaccgcgtttcagcagtggtatccgaaaagcctgcaggatgaagaaaaaccgcagatttataccggcctgtgggaatggaccagcaccgtgctgaaagaagatctggattttaccccggaagaactgtatccggattatacccgcgatttttttgatggcaaacataacgtggtgatgggcggcagctttaccaccgtggcgcgcattgcgaaccgccgcagctttcgcaacttttatcagcgcaaatatccgtatgcgtggattggcgcgcgcctggtgaaagtgaccaacaccctgagc

SEQ ID NO: 19 - protein, 426 aa, Taphrina deformans PYCC 5710
FSSNPRDIGPVPTLEEWSELWKLWDVITMEMVPREMLESKPIDLRNPCIFYVGHIPTFLDIHLSRVGNGRYLNPAYTQIFERGIDPDVDDPSQCHDHSSLPDKWPDLSEMLSFRDQVRKRLRDVYASGSINDRKVARAVFTVYEHEAMHIETFLYMHLQADWTLSPPKMLPPRFEEKPKEVGPASWMKMSPTTMNVGMNDVEGSDEGDYFGWDNEKPRRSTGLQPFTIQSRPVTNGEYAKYLNQTTEEGKRWRHPKSWTPDMRVKTPFGPIPLAAAVNWPVAASYDELEKYANWCGGRLPTHDELRHFIDSSCDTDDARGTPFNDVHGKKVNFSQWFPGNVEDSSKPQVYCGVWEWTSTPFARTPGFVTSQIYPGYSEDFFDGKHNIVLGGSWATISRIAARKSFVNWYQRNYEYAWTGCRLVKDV

SEQ ID NO: 20 - DNA, 1278 bp, Taphrina deformans PYCC 5710
  source 1..1278: mol_type = genomic DNA
tttagcagcaacccgcgcgatattggcccggtgccgaccctggaagaatggagcgaactgtggaaactgtgggatgtgattaccatggaaatggtgccgcgcgaaatgctggaaagcaaaccgattgatctgcgcaacccgtgcattttttatgtgggccatattccgacctttctggatattcatctgagccgcgtgggcaacggccgctatctgaacccggcgtatacccagatttttgaacgcggcattgatccggatgtggatgatccgagccagtgccatgatcatagcagcctgccggataaatggccggatctgagcgaaatgctgagctttcgcgatcaggtgcgcaaacgcctgcgcgatgtgtatgcgagcggcagcattaacgatcgcaaagtggcgcgcgcggtgtttaccgtgtatgaacatgaagcgatgcatattgaaacctttctgtatatgcatctgcaggcggattggaccctgagcccgccgaaaatgctgccgccgcgctttgaagaaaaaccgaaagaagtgggcccggcgagctggatgaaaatgagcccgaccaccatgaacgtgggcatgaacgatgtggaaggcagcgatgaaggcgattattttggctgggataacgaaaaaccgcgccgcagcaccggcctgcagccgtttaccattcagagccgcccggtgaccaacggcgaatatgcgaaatatctgaaccagaccaccgaagaaggcaaacgctggcgccatccgaaaagctggaccccggatatgcgcgtgaaaaccccgtttggcccgattccgctggcggcggcggtgaactggccggtggcggcgagctatgatgaactggaaaaatatgcgaactggtgcggcggccgcctgccgacccatgatgaactgcgccattttattgatagcagctgcgataccgatgatgcgcgcggcaccccgtttaacgatgtgcatggcaaaaaagtgaactttagccagtggtttccgggcaacgtggaagatagcagcaaaccgcaggtgtattgcggcgtgtgggaatggaccagcaccccgtttgcgcgcaccccgggctttgtgaccagccagatttatccgggctatagcgaagatttttttgatggcaaacataacattgtgctgggcggcagctgggcgaccattagccgcattgcggcgcgcaaaagctttgtgaactggtatcagcgcaactatgaatatgcgtggaccggctgccgcctggtgaaagatgtg

SEQ ID NO: 21 - protein, 422 aa, Protomyces lactucae-debilis
LSRQADTLKPVPSLAEWEQLWKLWDTITLGMIPQEMLLCKPIDLRHPCIFYLGHIPTFLDIHLTRVGNGKYTNDAYTRIFERGIDPDVDDPTHCHAHSDVPDTWPDLQEILAFRDTVRNRLREVYRQDTASFNRQLARALFVTFEHEAMHAETLLYMLLQSAETRPPPGVLSSLPTAAAPELEPAAWITLETSNFEVGMDDPEEAESGQYFGWDNEKPRRSISHAKVAIQARPISNGEYAAFLDAHPKLAAPASWTQSREVKTVFGPVPLTYAADWPVAASYDELQAYAKWKDARLPSFAELRHFLDDHSGESSNEPFNNVLDKNVNFGMWHPSSLTSSRESVQTYTGFWEWTSTEFSAPKGFVPSKVYPAYSSDFFDGKHNIVLGGSWATITRIAARKSFVNWYQRNYKFAWTSGRLARDL

SEQ ID NO: 22 - DNA, 1266 bp, Protomyces lactucae-debilis
  source 1..1266: mol_type = genomic DNA
ctgagccgccaggcggataccctgaaaccggtgccgagcctggcggaatgggaacagctgtggaaactgtgggataccattaccctgggcatgattccgcaggaaatgctgctgtgcaaaccgattgatctgcgccatccgtgcattttttatctgggccatattccgacctttctggatattcatctgacccgcgtgggcaacggcaaatataccaacgatgcgtatacccgcatttttgaacgcggcattgatccggatgtggatgatccgacccattgccatgcgcatagcgatgtgccggatacctggccggatctgcaggaaattctggcgtttcgcgataccgtgcgcaaccgcctgcgcgaagtgtatcgccaggataccgcgagctttaaccgccagctggcgcgcgcgctgtttgtgacctttgaacatgaagcgatgcatgcggaaaccctgctgtatatgctgctgcagagcgcggaaacccgcccgccgccgggcgtgctgagcagcctgccgaccgcggcggcgccggaactggaaccggcggcgtggattaccctggaaaccagcaactttgaagtgggcatggatgatccggaagaagcggaaagcggccagtattttggctgggataacgaaaaaccgcgccgcagcattagccatgcgaaagtggcgattcaggcgcgcccgattagcaacggcgaatatgcggcgtttctggatgcgcatccgaaactggcggcgccggcgagctggacccagagccgcgaagtgaaaaccgtgtttggcccggtgccgctgacctatgcggcggattggccggtggcggcgagctatgatgaactgcaggcgtatgcgaaatggaaagatgcgcgcctgccgagctttgcggaactgcgccattttctggatgatcatagcggcgaaagcagcaacgaaccgtttaacaacgtgctggataaaaacgtgaactttggcatgtggcatccgagcagcctgaccagcagccgcgaaagcgtgcagacctataccggcttttgggaatggaccagcaccgaatttagcgcgccgaaaggctttgtgccgagcaaagtgtatccggcgtatagcagcgatttttttgatggcaaacataacattgtgctgggcggcagctgggcgaccattacccgcattgcggcgcgcaaaagctttgtgaactggtatcagcgcaactataaatttgcgtggaccagcggccgcctggcgcgcgatctg

SEQ ID NO: 23 - protein, 468 aa, Saitoella complicata NRRL Y-17804
HIPLLGSKEPVPTTQDWSDLWSAWDTVTLQMIPQKMLLTKPIDLRHPCIFYIGHIPTFLDIHLTRAKLGGDAYINAAYTRIFERGIDPDVDDPTQCHVHSEVPDSWPDLQELLEFRDEVRARVKNCYGANGLVSSALDHVRRRALWLAFEHEAMHLETLLYMLLQSPQTVPPPGVPVPDWKLLASASQRPTATKEEDKWMMVESRKTNVGLNDPEGAENGGTDGRLMGWDNEKPQREWTVNGFIASKRPITNGEYATFLQESGSTKIPESWSRVDGVYKVKTVFGLVAMEHAHDWPVIGSYDEIASYATYAGGRLPREEELRALYDVIADSSATPGTLIAGVNGHLTSNGVHTTPPAVPNFIDLSGANVGFKHWHPTPAHATQLVGSGGVGAWEWTSTPMAPHEGFVPSKVYSGYTADFFDGKHNVVLGGSWATHGRLAGRRTFRNWYQRNYGFAWVTGRVIKDIDMN

SEQ ID NO: 24 - DNA, 1404 bp, Saitoella complicata NRRL Y-17804
  source 1..1404: mol_type = genomic DNA
catattccgctgctgggcagcaaagaaccggtgccgaccacccaggattggagcgatctgtggagcgcgtgggataccgtgaccctgcagatgattccgcagaaaatgctgctgaccaaaccgattgatctgcgccatccgtgcattttttatattggccatattccgacctttctggatattcatctgacccgcgcgaaactgggcggcgatgcgtatattaacgcggcgtatacccgcatttttgaacgcggcattgatccggatgtggatgatccgacccagtgccatgtgcatagcgaagtgccggatagctggccggatctgcaggaactgctggaatttcgcgatgaagtgcgcgcgcgcgtgaaaaactgctatggcgcgaacggcctggtgagcagcgcgctggatcatgtgcgccgccgcgcgctgtggctggcgtttgaacatgaagcgatgcatctggaaaccctgctgtatatgctgctgcagagcccgcagaccgtgccgccgccgggcgtgccggtgccggattggaaactgctggcgagcgcgagccagcgcccgaccgcgaccaaagaagaagataaatggatgatggtggaaagccgcaaaaccaacgtgggcctgaacgatccggaaggcgcggaaaacggcggcaccgatggccgcctgatgggctgggataacgaaaaaccgcagcgcgaatggaccgtgaacggctttattgcgagcaaacgcccgattaccaacggcgaatatgcgacctttctgcaggaaagcggcagcaccaaaattccggaaagctggagccgcgtggatggcgtgtataaagtgaaaaccgtgtttggcctggtggcgatggaacatgcgcatgattggccggtgattggcagctatgatgaaattgcgagctatgcgacctatgcgggcggccgcctgccgcgcgaagaagaactgcgcgcgctgtatgatgtgattgcggatagcagcgcgaccccgggcaccctgattgcgggcgtgaacggccatctgaccagcaacggcgtgcataccaccccgccggcggtgccgaactttattgatctgagcggcgcgaacgtgggctttaaacattggcatccgaccccggcgcatgcgacccagctggtgggcagcggcggcgtgggcgcgtgggaatggaccagcaccccgatggcgccgcatgaaggctttgtgccgagcaaagtgtatagcggctataccgcggatttttttgatggcaaacataacgtggtgctgggcggcagctgggcgacccatggccgcctggcgggccgccgcacctttcgcaactggtatcagcgcaactatggctttgcgtgggtgaccggccgcgtgattaaagatattgatatgaac

SEQ ID NO: 25 - protein, 463 aa, Tortispora caseinolytica NRRL Y-17796
HLVYKPECRLPLASVVANMPSLEEWAYMHNMWDYVTCKMAPESMYLEQPIYLRNTVIFYLGHSPCFLDVVLNRANTGTLATQPVWYQDIFARGIDPDVDDPSKVHSHSSIPAEWPPLDDILQYQDSVRSRLRRLLTDNTGKMSSRTARAIWLGYEHDAMHLETLMYMMLQSPLKLSPPGVPKPSFIQSKHANSNQKWIRIPATVINIGIDDPDEADHRPGSHASRLMGWDNEKPSRGSVTVPPFSASPSLITNRQYYSYLLDRLRSGVVIKPPESWNASEDLQNVYVKTFFGDAPLCVDGSLNSDFIASDWPVCASYNELQEFMAQFQNGEFRFPTEHEVLAIYKTQQQRLHNDDPDYYDLSDSNVGFKHWHPSSNVDCIEGISGPGGQGVWEWTSTVFDSHEGFTVNELYPEYSADFFDGKHNVVLGGSWATAPRLSGRRSFRNWYQRSYCFAWIGARMVRK

SEQ ID NO: 26 - DNA, 1389 bp, Tortispora caseinolytica NRRL Y-17796
  source 1..1389: mol_type = genomic DNA
catctggtgtataaaccggaatgccgcctgccgctggcgagcgtggtggcgaacatgccgagcctggaagaatgggcgtatatgcataacatgtgggattatgtgacctgcaaaatggcgccggaaagcatgtatctggaacagccgatttatctgcgcaacaccgtgattttttatctgggccatagcccgtgctttctggatgtggtgctgaaccgcgcgaacaccggcaccctggcgacccagccggtgtggtatcaggatatttttgcgcgcggcattgatccggatgtggatgatccgagcaaagtgcatagccatagcagcattccggcggaatggccgccgctggatgatattctgcagtatcaggatagcgtgcgcagccgcctgcgccgcctgctgaccgataacaccggcaaaatgagcagccgcaccgcgcgcgcgatttggctgggctatgaacatgatgcgatgcatctggaaaccctgatgtatatgatgctgcagagcccgctgaaactgagcccgccgggcgtgccgaaaccgagctttattcagagcaaacatgcgaacagcaaccagaaatggattcgcattccggcgaccgtgattaacattggcattgatgatccggatgaagcggatcatcgcccgggcagccatgcgagccgcctgatgggctgggataacgaaaaaccgagccgcggcagcgtgaccgtgccgccgtttagcgcgagcccgagcctgattaccaaccgccagtattatagctatctgctggatcgcctgcgcagcggcgtggtgattaaaccgccggaaagctggaacgcgagcgaagatctgcagaacgtgtatgtgaaaaccttttttggcgatgcgccgctgtgcgtggatggcagcctgaacagcgattttattgcgagcgattggccggtgtgcgcgagctataacgaactgcaggaatttatggcgcagtttcagaacggcgaatttcgctttccgaccgaacatgaagtgctggcgatttataaaacccagcagcagcgcctgcataacgatgatccggattattatgatctgagcgatagcaacgtgggctttaaacattggcatccgagcagcaacgtggattgcattgaaggcattagcggcccgggcggccagggcgtgtgggaatggaccagcaccgtgtttgatagccatgaaggctttaccgtgaacgaactgtatccggaatatagcgcggatttttttgatggcaaacataacgtggtgctgggcggcagctgggcgaccgcgccgcgcctgagcggccgccgcagctttcgcaactggtatcagcgcagctattgctttgcgtggattggcgcgcgcatggtgcgcaaa

SEQ ID NO: 27 - protein, 519 aa, Neurospora crassa
FSLIPSVYARSALPTLDDWEALWATWDVVTRQMLPQEELLEKPIKLRNACIFYLGHIPTFLDIQLTKTTKQAPSEPAHFCKIFERGIDPDVDNPELCHAHSEIPDEWPPVEEILTYQETVRSRLRGLYAHGIANIPRNVGRAIWVGFEHELMHIETLLYMMLQSDKTLIPTHIPRPDFDKLARKAESERVPNQWFKIPAQEITIGLDDPEDGSDINKHYGWDNEKPPRRVQVAAFQAQGRPITNEEYAQYLLEKNIDKLPASWARLDNENISNGTTNSVSGHHSNRTSKQQLPSSFLEKTAVRTVYGLVPLKHALDWPVFASYDELAGCAAYMGGRIPTFEETRSIYAYADALKKKKEAERQLGRTVPAVNAHLTNNGVEITPPSSPSSETPAESSSPSDSNTTLITTEDLFSDLDGANVGFHNWHPMPITSKGNTLVGQGELGGVWEWTSSVLRKWEGFEPMELYPGYTADFFDEKHNIVLGGSWATHPRIAGRKSFVNWYQRNYPYAWVGARVVRDL

SEQ ID NO: 28 - DNA, 1557 bp, Neurospora crassa
  source 1..1557: mol_type = genomic DNA
tttagcctgattccgagcgtgtatgcgcgcagcgcgctgccgaccctggatgattgggaagcgctgtgggcgacctgggatgtggtgacccgccagatgctgccgcaggaagaactgctggaaaaaccgattaaactgcgcaacgcgtgcattttttatctgggccatattccgacctttctggatattcagctgaccaaaaccaccaaacaggcgccgagcgaaccggcgcatttttgcaaaatttttgaacgcggcattgatccggatgtggataacccggaactgtgccatgcgcatagcgaaattccggatgaatggccgccggtggaagaaattctgacctatcaggaaaccgtgcgcagccgcctgcgcggcctgtatgcgcatggcattgcgaacattccgcgcaacgtgggccgcgcgatttgggtgggctttgaacatgaactgatgcatattgaaaccctgctgtatatgatgctgcagagcgataaaaccctgattccgacccatattccgcgcccggattttgataaactggcgcgcaaagcggaaagcgaacgcgtgccgaaccagtggtttaaaattccggcgcaggaaattaccattggcctggatgatccggaagatggcagcgatattaacaaacattatggctgggataacgaaaaaccgccgcgccgcgtgcaggtggcggcgtttcaggcgcagggccgcccgattaccaacgaagaatatgcgcagtatctgctggaaaaaaacattgataaactgccggcgagctgggcgcgcctggataacgaaaacattagcaacggcaccaccaacagcgtgagcggccatcatagcaaccgcaccagcaaacagcagctgccgagcagctttctggaaaaaaccgcggtgcgcaccgtgtatggcctggtgccgctgaaacatgcgctggattggccggtgtttgcgagctatgatgaactggcgggctgcgcggcgtatatgggcggccgcattccgacctttgaagaaacccgcagcatttatgcgtatgcggatgcgctgaaaaaaaaaaaagaagcggaacgccagctgggccgcaccgtgccggcggtgaacgcgcatctgaccaacaacggcgtggaaattaccccgccgagcagcccgagcagcgaaaccccggcggaaagcagcagcccgagcgatagcaacaccaccctgattaccaccgaagatctgtttagcgatctggatggcgcgaacgtgggctttcataactggcatccgatgccgattaccagcaaaggcaacaccctggtgggccagggcgaactgggcggcgtgtgggaatggaccagcagcgtgctgcgcaaatgggaaggctttgaaccgatggaactgtatccgggctataccgcggatttttttgatgaaaaacataacattgtgctgggcggcagctgggcgacccatccgcgcattgcgggccgcaaaagctttgtgaactggtatcagcgcaactatccgtatgcgtgggtgggcgcgcgcgtggtgcgcgatctg

SEQ ID NO: 29 - protein, 392 aa, Schizosaccharomyces cryophilus OY26
MSDCMPFGHALKPYYMLDKNYVSVNNGSYGVVCASAFQRHLQLLEESEKTQDLQMKYRLPKLANNTLLQIAELLDTTSSNLAFCFSATQAISSILLTFPWSANDKILSLNVAYPTCQFALDFVRNRYDVQVDTLEVEFIYDPSEFLSRVESYLVKNKPRVFIFDFITSMPVTQLPCKELIQLCKKYGVISVVDAAHGIGFCPLSLSSLDPDFLYTNAHKWLNAPSGTTILYVSKKYHNFIEALPISYGYHIRKQNSPPADSLGIRFLNASFMDLPKFIAIDAAIAFRKSIGGEHKIQSYNHDIAVRGSKIIAESLGTSYFALASPIAMVNVEVPLRCIPSADFLEEFWQSKNTFLRFVEYQGRYYTRVGGAPFLEESDFVYVADVLKELCQK

SEQ ID NO: 30 - DNA, 1176 bp, Schizosaccharomyces cryophilus OY26
  source 1..1176: mol_type = genomic DNA
atgagcgattgcatgccgtttggccatgcgctgaaaccgtattatatgctggataaaaactatgtgagcgtgaacaacggcagctatggcgtggtgtgcgcgagcgcgtttcagcgccatctgcagctgctggaagaaagcgaaaaaacccaggatctgcagatgaaatatcgcctgccgaaactggcgaacaacaccctgctgcagattgcggaactgctggataccaccagcagcaacctggcgttttgctttagcgcgacccaggcgattagcagcattctgctgacctttccgtggagcgcgaacgataaaattctgagcctgaacgtggcgtatccgacctgccagtttgcgctggattttgtgcgcaaccgctatgatgtgcaggtggataccctggaagtggaatttatttatgatccgagcgaatttctgagccgcgtggaaagctatctggtgaaaaacaaaccgcgcgtgtttatttttgattttattaccagcatgccggtgacccagctgccgtgcaaagaactgattcagctgtgcaaaaaatatggcgtgattagcgtggtggatgcggcgcatggcattggcttttgcccgctgagcctgagcagcctggatccggattttctgtataccaacgcgcataaatggctgaacgcgccgagcggcaccaccattctgtatgtgagcaaaaaatatcataactttattgaagcgctgccgattagctatggctatcatattcgcaaacagaacagcccgccggcggatagcctgggcattcgctttctgaacgcgagctttatggatctgccgaaatttattgcgattgatgcggcgattgcgtttcgcaaaagcattggcggcgaacataaaattcagagctataaccatgatattgcggtgcgcggcagcaaaattattgcggaaagcctgggcaccagctattttgcgctggcgagcccgattgcgatggtgaacgtggaagtgccgctgcgctgcattccgagcgcggattttctggaagaattttggcagagcaaaaacacctttctgcgctttgtggaatatcagggccgctattatacccgcgtgggcggcgcgccgtttctggaagaaagcgattttgtgtatgtggcggatgtgctgaaagaactgtgccagaaa

SEQ ID NO: 31 - protein, 396 aa, Schizosaccharomyces octosporus yFS286
MSQEVPFGHALTRHFMLDENYVSVNNASCGVVCVPAFQQHIRLLEESEKVQDLQTRYRLPKLAEQTLNQIAELLDTSPSNLAFCFSATQAISSILLTFPWTPNDRILTLNLAYPTCQFAVDFVRDRHGIQVDTIDIDLAYNRLELLSQIESYLEKNKPRVFVFDFVTSMPVVQLPCKEIVQICKKYNVISVIDAAHGIGLCPLSLSSLDPDFLYTNAHKWLNAPSGTTILYVSEKYHDSIEALPISYGYHIRKENSPPADALNVRFLYASSTDLPKYIAIKDAIAFRKSIGGEHKIQSYNYQIAIKGAKIIAEALGTSYFALAPPIAMVNVEIPLRCIPSSSFLEEFWQKKNTFLRFVKYHGKIYTRIAGAPFLEESDFLYTVDVLKELCQFSHES

SEQ ID NO: 32 - DNA, 1188 bp, Schizosaccharomyces octosporus yFS286
  source 1..1188: mol_type = genomic DNA
atgagccaggaagtgccgtttggccatgcgctgacccgccattttatgctggatgaaaactatgtgagcgtgaacaacgcgagctgcggcgtggtgtgcgtgccggcgtttcagcagcatattcgcctgctggaagaaagcgaaaaagtgcaggatctgcagacccgctatcgcctgccgaaactggcggaacagaccctgaaccagattgcggaactgctggataccagcccgagcaacctggcgttttgctttagcgcgacccaggcgattagcagcattctgctgacctttccgtggaccccgaacgatcgcattctgaccctgaacctggcgtatccgacctgccagtttgcggtggattttgtgcgcgatcgccatggcattcaggtggataccattgatattgatctggcgtataaccgcctggaactgctgagccagattgaaagctatctggaaaaaaacaaaccgcgcgtgtttgtgtttgattttgtgaccagcatgccggtggtgcagctgccgtgcaaagaaattgtgcagatttgcaaaaaatataacgtgattagcgtgattgatgcggcgcatggcattggcctgtgcccgctgagcctgagcagcctggatccggattttctgtataccaacgcgcataaatggctgaacgcgccgagcggcaccaccattctgtatgtgagcgaaaaatatcatgatagcattgaagcgctgccgattagctatggctatcatattcgcaaagaaaacagcccgccggcggatgcgctgaacgtgcgctttctgtatgcgagcagcaccgatctgccgaaatatattgcgattaaagatgcgattgcgtttcgcaaaagcattggcggcgaacataaaattcagagctataactatcagattgcgattaaaggcgcgaaaattattgcggaagcgctgggcaccagctattttgcgctggcgccgccgattgcgatggtgaacgtggaaattccgctgcgctgcattccgagcagcagctttctggaagaattttggcagaaaaaaaacacctttctgcgctttgtgaaatatcatggcaaaatttatacccgcattgcgggcgcgccgtttctggaagaaagcgattttctgtataccgtggatgtgctgaaagaactgtgccagtttagccatgaaagc

SEQ ID NO: 33 - protein, 396 aa, Schizosaccharomyces osmophilus
MSECIPFGRALKPYFMLDEKYVSVNNASSGVVCVPAFQRHLQLLEESEKVQDLQTRYRLPKLAEKTMDQLAELLDTSPNNLAFCFSATQAISSILLTFPWIANDRILTLNLAYPTCQFAVDFVQDRYDVQMDTIDIDFAYDRSELLSRVESYLAKNKPRLFIFDFVTSMPVIQLPCKELIQLCKKYNVISVIDAAHGIGLSPLSMSSLDPDFLYTNAHKWLNAPSGTTILYVSKKYHNSIEALPISYGYHIRKQKSPPPAPLNARFLYASSTDLPKFIAIDAAIAFRKSIGGEHKIQNYNYDIIIKGAKIIAEALGTSYFVLAPPIAMVNVEIPLRRMPSAEFFEYFWQSKNTFLRFVEYHGKFYTRIAGAPFLEESDFVYIAGVLKELCQNSPEN

SEQ ID NO: 34 - DNA, 1188 bp, Schizosaccharomyces osmophilus
  source 1..1188: mol_type = genomic DNA
atgagcgaatgcattccgtttggccgcgcgctgaaaccgtattttatgctggatgaaaaatatgtgagcgtgaacaacgcgagcagcggcgtggtgtgcgtgccggcgtttcagcgccatctgcagctgctggaagaaagcgaaaaagtgcaggatctgcagacccgctatcgcctgccgaaactggcggaaaaaaccatggatcagctggcggaactgctggataccagcccgaacaacctggcgttttgctttagcgcgacccaggcgattagcagcattctgctgacctttccgtggattgcgaacgatcgcattctgaccctgaacctggcgtatccgacctgccagtttgcggtggattttgtgcaggatcgctatgatgtgcagatggataccattgatattgattttgcgtatgatcgcagcgaactgctgagccgcgtggaaagctatctggcgaaaaacaaaccgcgcctgtttatttttgattttgtgaccagcatgccggtgattcagctgccgtgcaaagaactgattcagctgtgcaaaaaatataacgtgattagcgtgattgatgcggcgcatggcattggcctgagcccgctgagcatgagcagcctggatccggattttctgtataccaacgcgcataaatggctgaacgcgccgagcggcaccaccattctgtatgtgagcaaaaaatatcataacagcattgaagcgctgccgattagctatggctatcatattcgcaaacagaaaagcccgccgccggcgccgctgaacgcgcgctttctgtatgcgagcagcaccgatctgccgaaatttattgcgattgatgcggcgattgcgtttcgcaaaagcattggcggcgaacataaaattcagaactataactatgatattattattaaaggcgcgaaaattattgcggaagcgctgggcaccagctattttgtgctggcgccgccgattgcgatggtgaacgtggaaattccgctgcgccgcatgccgagcgcggaattttttgaatatttttggcagagcaaaaacacctttctgcgctttgtggaatatcatggcaaattttatacccgcattgcgggcgcgccgtttctggaagaaagcgattttgtgtatattgcgggcgtgctgaaagaactgtgccagaacagcccggaaaac

SEQ ID NO: 35 - protein, 395 aa, Schizosaccharomyces japonicus yFS275
MEGKDSKAVVFGHALKKEFFVDDNVVCANTGSFGTVCRQAFAATEEAVKVSQKNTDLGFLYELPRRMRRLRSRVAEFVGAKESDIAFVGTATHAVSTILLTHPWKQGDRLLMLSLAYPTCSFAADYVRDRYGVEIELIDVDVDFDGEEFLKTVRERFEAFRPKMFLFDLISSMPVVLTPWEKVVELCREYNVLSVVDGAHSVGLLDLNLDKVQPDFFFTNTHKWLFAPSGTTILYVSEKNHSLIDPLPLSYGYGYRKEDAKPAAPFAERFRFSTYMDSAKYLGIEGALDFRATLGEEAIRRYTNEIANKGAKIVADALGVPFTPAPFPLSMVNVELPIKEVPALATEEFWKKHNTFVRTCEYKGKWYTRICGCIFMEESDYERVAVALKELCGVN

SEQ ID NO: 36 - DNA, 1185 bp, Schizosaccharomyces japonicus yFS275
  source 1..1185: mol_type = genomic DNA
atggaaggcaaagatagcaaagcggtggtgtttggccatgcgctgaaaaaagaattttttgtggatgataacgtggtgtgcgcgaacaccggcagctttggcaccgtgtgccgccaggcgtttgcggcgaccgaagaagcggtgaaagtgagccagaaaaacaccgatctgggctttctgtatgaactgccgcgccgcatgcgccgcctgcgcagccgcgtggcggaatttgtgggcgcgaaagaaagcgatattgcgtttgtgggcaccgcgacccatgcggtgagcaccattctgctgacccatccgtggaaacagggcgatcgcctgctgatgctgagcctggcgtatccgacctgcagctttgcggcggattatgtgcgcgatcgctatggcgtggaaattgaactgattgatgtggatgtggattttgatggcgaagaatttctgaaaaccgtgcgcgaacgctttgaagcgtttcgcccgaaaatgtttctgtttgatctgattagcagcatgccggtggtgctgaccccgtgggaaaaagtggtggaactgtgccgcgaatataacgtgctgagcgtggtggatggcgcgcatagcgtgggcctgctggatctgaacctggataaagtgcagccggattttttttttaccaacacccataaatggctgtttgcgccgagcggcaccaccattctgtatgtgagcgaaaaaaaccatagcctgattgatccgctgccgctgagctatggctatggctatcgcaaagaagatgcgaaaccggcggcgccgtttgcggaacgctttcgctttagcacctatatggatagcgcgaaatatctgggcattgaaggcgcgctggattttcgcgcgaccctgggcgaagaagcgattcgccgctataccaacgaaattgcgaacaaaggcgcgaaaattgtggcggatgcgctgggcgtgccgtttaccccggcgccgtttccgctgagcatggtgaacgtggaactgccgattaaagaagtgccggcgctggcgaccgaagaattttggaaaaaacataacacctttgtgcgcacctgcgaatataaaggcaaatggtatacccgcatttgcggctgcatttttatggaagaaagcgattatgaacgcgtggcggtggcgctgaaagaactgtgcggcgtgaac

SEQ ID NO: 37 - protein, 406 aa, Mucor lusitanicus
MGSLFGKSLRSQFLLEPQYTSLNHGSYGSIPRALLPVLDELRLKSEVNPDRWLRREMFPVIEKNKRVVADLVHVDPQELVFVFNAMTGINTVARSLPLEAGDKILYFNTAYNSVESTIKFIKNSEKLKLIRIDLAYPLDDSEVLAKMQETIERESSKGDGNIKLCFMDAISSVPAVRFPFESAVKLVREHNILSLVDGAHAIGQIPLDLHQVDPDFFITNCHKWLYAPRGCAVLYVPFRNQRMIHPAIINSAYADHSDPADKSVSFQDEFAWPGTADFSNFMCIEAAVEFRKSIGGEDAIMTYCHELAAKGGEIAANILGTQVMGNPGQIAMVNVEIPLTNTKLSDAQIIGIFIDKLLYEHNCMAPVYKHNGIWHTRLSAQVYNDESDFETVAKAILAVCQELNKD

SEQ ID NO: 38 - DNA, 1218 bp, Mucor lusitanicus
  source 1..1218: mol_type = genomic DNA
atgggcagcctgtttggcaaaagcctgcgcagccagtttctgctggaaccgcagtataccagcctgaaccatggcagctatggcagcattccgcgcgcgctgctgccggtgctggatgaactgcgcctgaaaagcgaagtgaacccggatcgctggctgcgccgcgaaatgtttccggtgattgaaaaaaacaaacgcgtggtggcggatctggtgcatgtggatccgcaggaactggtgtttgtgtttaacgcgatgaccggcattaacaccgtggcgcgcagcctgccgctggaagcgggcgataaaattctgtattttaacaccgcgtataacagcgtggaaagcaccattaaatttattaaaaacagcgaaaaactgaaactgattcgcattgatctggcgtatccgctggatgatagcgaagtgctggcgaaaatgcaggaaaccattgaacgcgaaagcagcaaaggcgatggcaacattaaactgtgctttatggatgcgattagcagcgtgccggcggtgcgctttccgtttgaaagcgcggtgaaactggtgcgcgaacataacattctgagcctggtggatggcgcgcatgcgattggccagattccgctggatctgcatcaggtggatccggatttttttattaccaactgccataaatggctgtatgcgccgcgcggctgcgcggtgctgtatgtgccgtttcgcaaccagcgcatgattcatccggcgattattaacagcgcgtatgcggatcatagcgatccggcggataaaagcgtgagctttcaggatgaatttgcgtggccgggcaccgcggattttagcaactttatgtgcattgaagcggcggtggaatttcgcaaaagcattggcggcgaagatgcgattatgacctattgccatgaactggcggcgaaaggcggcgaaattgcggcgaacattctgggcacccaggtgatgggcaacccgggccagattgcgatggtgaacgtggaaattccgctgaccaacaccaaactgagcgatgcgcagattattggcatttttattgataaactgctgtatgaacataactgcatggcgccggtgtataaacataacggcatttggcatacccgcctgagcgcgcaggtgtataacgatgaaagcgattttgaaaccgtggcgaaagcgattctggcggtgtgccaggaactgaacaaagat

SEQ ID NO: 39 - protein, 409 aa, Mucor lusitanicus CBS 277.49
MTQGTTQFGKSLRSQFLLEPQYTSLNHGSYGSIPRALLPVLDELRLKSEVNPDRWLRREMFPVIEKNKRVVADLVHVDPQELVFVFNAMTGINTVARSLPLEAGDKILYFNTAYNSVESTIKFIKNSEKLKLIRIDLAYPLDDSEVLAKMQETIERESSKGDGNIKLCFMDAISSVPAVRFPFESAVKLVREHNILSLVDGAHAIGQIPLDLHQVDPDFFITNCHKWLYAPRGCAVLYVPFRNQRMIHPAIINSAYADHSDPADKSVSFQDEFAWPGTADFSNFMCIEAAVEFRKSIGGEDAIMTYCHELAAKGGEIAANILGTQVMGNPGQIAMVNVEIPLTNTKLSDAQIIGIFIDKLLYEHNCMAPVYKHNGIWHTRLSAQVYNDESDFETVAKAILAVCQELNKD

SEQ ID NO: 40 - DNA, 1227 bp, Mucor lusitanicus CBS 277.49
  source 1..1227: mol_type = genomic DNA
atgacccagggcaccacccagtttggcaaaagcctgcgcagccagtttctgctggaaccgcagtataccagcctgaaccatggcagctatggcagcattccgcgcgcgctgctgccggtgctggatgaactgcgcctgaaaagcgaagtgaacccggatcgctggctgcgccgcgaaatgtttccggtgattgaaaaaaacaaacgcgtggtggcggatctggtgcatgtggatccgcaggaactggtgtttgtgtttaacgcgatgaccggcattaacaccgtggcgcgcagcctgccgctggaagcgggcgataaaattctgtattttaacaccgcgtataacagcgtggaaagcaccattaaatttattaaaaacagcgaaaaactgaaactgattcgcattgatctggcgtatccgctggatgatagcgaagtgctggcgaaaatgcaggaaaccattgaacgcgaaagcagcaaaggcgatggcaacattaaactgtgctttatggatgcgattagcagcgtgccggcggtgcgctttccgtttgaaagcgcggtgaaactggtgcgcgaacataacattctgagcctggtggatggcgcgcatgcgattggccagattccgctggatctgcatcaggtggatccggatttttttattaccaactgccataaatggctgtatgcgccgcgcggctgcgcggtgctgtatgtgccgtttcgcaaccagcgcatgattcatccggcgattattaacagcgcgtatgcggatcatagcgatccggcggataaaagcgtgagctttcaggatgaatttgcgtggccgggcaccgcggattttagcaactttatgtgcattgaagcggcggtggaatttcgcaaaagcattggcggcgaagatgcgattatgacctattgccatgaactggcggcgaaaggcggcgaaattgcggcgaacattctgggcacccaggtgatgggcaacccgggccagattgcgatggtgaacgtggaaattccgctgaccaacaccaaactgagcgatgcgcagattattggcatttttattgataaactgctgtatgaacataactgcatggcgccggtgtataaacataacggcatttggcatacccgcctgagcgcgcaggtgtataacgatgaaagcgattttgaaaccgtggcgaaagcgattctggcggtgtgccaggaactgaacaaagat

SEQ ID NO: 41 - protein, 409 aa, Mucor circinelloides 1006PhL
MTQGTAQFGRNLRSQFLLEPQYTSLNHGSYGSIPRALLPVLEDLRLKSEVNPDRWLRREMFPVIERNKKVVADLVHVDPQELVFVFNAMTGINTVARSLPLEAGDKVIYFNTAYNSVESTIKFIKNSEKLKLIRIDLAYPLDDNQVLTILQETIERENSRGDGTIKLCFMDAISSVPAVRFPFESAVKLVREHNILSLVDGAHAIGQIPLDLHQVDPDFFITNCHKWLYAPRGCAILYVPFRNQRLIHPAIINSAYADHSDPADKSVSFQDEFAWPGTADFSNFMCIEAAVEFRKSLGGEDAIMAYCHDLAIKGGAIAAEILGTKVMENTGQIAMVNVEIPLGNTELSDAQIIGIFIDKLLYEHNCMAPVYKHNNIWYTRLSAQVYNDESDFETVAKAILAVCQELDRD

SEQ ID NO: 42 - DNA, 1227 bp, Mucor circinelloides 1006PhL
  source 1..1227: mol_type = genomic DNA
atgacccagggcaccgcgcagtttggccgcaacctgcgcagccagtttctgctggaaccgcagtataccagcctgaaccatggcagctatggcagcattccgcgcgcgctgctgccggtgctggaagatctgcgcctgaaaagcgaagtgaacccggatcgctggctgcgccgcgaaatgtttccggtgattgaacgcaacaaaaaagtggtggcggatctggtgcatgtggatccgcaggaactggtgtttgtgtttaacgcgatgaccggcattaacaccgtggcgcgcagcctgccgctggaagcgggcgataaagtgatttattttaacaccgcgtataacagcgtggaaagcaccattaaatttattaaaaacagcgaaaaactgaaactgattcgcattgatctggcgtatccgctggatgataaccaggtgctgaccattctgcaggaaaccattgaacgcgaaaacagccgcggcgatggcaccattaaactgtgctttatggatgcgattagcagcgtgccggcggtgcgctttccgtttgaaagcgcggtgaaactggtgcgcgaacataacattctgagcctggtggatggcgcgcatgcgattggccagattccgctggatctgcatcaggtggatccggatttttttattaccaactgccataaatggctgtatgcgccgcgcggctgcgcgattctgtatgtgccgtttcgcaaccagcgcctgattcatccggcgattattaacagcgcgtatgcggatcatagcgatccggcggataaaagcgtgagctttcaggatgaatttgcgtggccgggcaccgcggattttagcaactttatgtgcattgaagcggcggtggaatttcgcaaaagcctgggcggcgaagatgcgattatggcgtattgccatgatctggcgattaaaggcggcgcgattgcggcggaaattctgggcaccaaagtgatggaaaacaccggccagattgcgatggtgaacgtggaaattccgctgggcaacaccgaactgagcgatgcgcagattattggcatttttattgataaactgctgtatgaacataactgcatggcgccggtgtataaacataacaacatttggtatacccgcctgagcgcgcaggtgtataacgatgaaagcgattttgaaaccgtggcgaaagcgattctggcggtgtgccaggaactggatcgcgat

SEQ ID NO: 43 - protein, 412 aa, Thamnidium elegans
MNNTTAPELGRNIREQFLFEPGYISLNHGSYGSIPKMLVPVLQDLRMKAEVNPDRWLRREMFPEIDKNRNTLANLVHADPQELVFVFNAMTGINTVARSLPLEAGDKILYFNTAYNSVESTIKFVKNYEQLKLVKIDLAYPMSDSEVLDLIEETIEKENQKNDGTIKVCFMDAISSVPAVLFPFESAIKLVRKHNILSMVDGAHAIGQIPLDLHEMDPDFFITNCHKWLYAPRGCAVLYVPSRNQRLIHPAIINSDYADHSDPSDKTNTFQKEFAWPGTSDFSNFMSINSAMEFRRSLGGEEAIMKYTRDLAVKGGEVAAKILDTDIMENAEKTLTVAMVNVRLPLKKPNVSDVEVVQVFIDKLLNEHNCMAPVYKHNDIWYTRLSAQVYNDVTDFEYVAKAILSVCKELES

SEQ ID NO: 44 - DNA, 1236 bp, Thamnidium elegans
  source 1..1236: mol_type = genomic DNA
atgaacaacaccaccgcgccggaactgggccgcaacattcgcgaacagtttctgtttgaaccgggctatattagcctgaaccatggcagctatggcagcattccgaaaatgctggtgccggtgctgcaggatctgcgcatgaaagcggaagtgaacccggatcgctggctgcgccgcgaaatgtttccggaaattgataaaaaccgcaacaccctggcgaacctggtgcatgcggatccgcaggaactggtgtttgtgtttaacgcgatgaccggcattaacaccgtggcgcgcagcctgccgctggaagcgggcgataaaattctgtattttaacaccgcgtataacagcgtggaaagcaccattaaatttgtgaaaaactatgaacagctgaaactggtgaaaattgatctggcgtatccgatgagcgatagcgaagtgctggatctgattgaagaaaccattgaaaaagaaaaccagaaaaacgatggcaccattaaagtgtgctttatggatgcgattagcagcgtgccggcggtgctgtttccgtttgaaagcgcgattaaactggtgcgcaaacataacattctgagcatggtggatggcgcgcatgcgattggccagattccgctggatctgcatgaaatggatccggatttttttattaccaactgccataaatggctgtatgcgccgcgcggctgcgcggtgctgtatgtgccgagccgcaaccagcgcctgattcatccggcgattattaacagcgattatgcggatcatagcgatccgagcgataaaaccaacacctttcagaaagaatttgcgtggccgggcaccagcgattttagcaactttatgagcattaacagcgcgatggaatttcgccgcagcctgggcggcgaagaagcgattatgaaatatacccgcgatctggcggtgaaaggcggcgaagtggcggcgaaaattctggataccgatattatggaaaacgcggaaaaaaccctgaccgtggcgatggtgaacgtgcgcctgccgctgaaaaaaccgaacgtgagcgatgtggaagtggtgcaggtgtttattgataaactgctgaacgaacataactgcatggcgccggtgtataaacataacgatatttggtatacccgcctgagcgcgcaggtgtataacgatgtgaccgattttgaatatgtggcgaaagcgattctgagcgtgtgcaaagaactggaaagc

SEQ ID NO: 45 - protein, 473 aa, Neurospora crassa
MVATTVELPLQQKADAAQTVTGPLPFGNSLLKEFVLDPAYRNLNHGSFGTIPSAIQQKLRSYQTAAEARPCPFLRYQTPVLLDESRAAVANLLKVPVETVVFVANATMGVNTVLRNIVWSADGKDEILYFDTIYGACGKTIDYVIEDKRGIVSSRCIPLIYPAEDDDVVAAFRDAIKKSREEGKRPRLAVIDVVSSMPGVRFPFEDIVKICKEEEIISCVDGAQGIGMVDLKITETDPDFLISNCHKWLFTPRGCAVFYVPVRNQHLIRSTLPTSHGFVPQVGNRFNPLVPAGNKSAFVSNFEFVGTVDNSPFFCVKDAIKWREEVLGGEERIMEYMTKLAREGGQKVAEILGTRVLENSTGTLIRCAMVNIALPFVVGEDPKAPVKLTEKEEKDVEGLYEIPHEEANMAFKWMYNVLQDEFNTFVPMTFHRRRFWARLSAQVYLEMSDFEWAGKTLKELCERVAKGEYKESA

SEQ ID NO: 46 - DNA, 1419 bp, Neurospora crassa
  source 1..1419: mol_type = genomic DNA
atggtggcgaccaccgtggaactgccgctgcagcagaaagcggatgcggcgcagaccgtgaccggcccgctgccgtttggcaacagcctgctgaaagaatttgtgctggatccggcgtatcgcaacctgaaccatggcagctttggcaccattccgagcgcgattcagcagaaactgcgcagctatcagaccgcggcggaagcgcgcccgtgcccgtttctgcgctatcagaccccggtgctgctggatgaaagccgcgcggcggtggcgaacctgctgaaagtgccggtggaaaccgtggtgtttgtggcgaacgcgaccatgggcgtgaacaccgtgctgcgcaacattgtgtggagcgcggatggcaaagatgaaattctgtattttgataccatttatggcgcgtgcggcaaaaccattgattatgtgattgaagataaacgcggcattgtgagcagccgctgcattccgctgatttatccggcggaagatgatgatgtggtggcggcgtttcgcgatgcgattaaaaaaagccgcgaagaaggcaaacgcccgcgcctggcggtgattgatgtggtgagcagcatgccgggcgtgcgctttccgtttgaagatattgtgaaaatttgcaaagaagaagaaattattagctgcgtggatggcgcgcagggcattggcatggtggatctgaaaattaccgaaaccgatccggattttctgattagcaactgccataaatggctgtttaccccgcgcggctgcgcggtgttttatgtgccggtgcgcaaccagcatctgattcgcagcaccctgccgaccagccatggctttgtgccgcaggtgggcaaccgctttaacccgctggtgccggcgggcaacaaaagcgcgtttgtgagcaactttgaatttgtgggcaccgtggataacagcccgtttttttgcgtgaaagatgcgattaaatggcgcgaagaagtgctgggcggcgaagaacgcattatggaatatatgaccaaactggcgcgcgaaggcggccagaaagtggcggaaattctgggcacccgcgtgctggaaaacagcaccggcaccctgattcgctgcgcgatggtgaacattgcgctgccgtttgtggtgggcgaagatccgaaagcgccggtgaaactgaccgaaaaagaagaaaaagatgtggaaggcctgtatgaaattccgcatgaagaagcgaacatggcgtttaaatggatgtataacgtgctgcaggatgaatttaacacctttgtgccgatgacctttcatcgccgccgcttttgggcgcgcctgagcgcgcaggtgtatctggaaatgagcgattttgaatgggcgggcaaaaccctgaaagaactgtgcgaacgcgtggcgaaaggcgaatataaagaaagcgcg

SEQ ID NO: 47 - DNA, 26 bp, synthetic construct
  misc_feature 1..26: note = Spegt1-tr F1
  source 1..26: mol_type = other DNA
ggacaatatgtacaccgcctggattc

SEQ ID NO: 48 - DNA, 27 bp, synthetic construct
  misc_feature 1..27: note = Spegt1-tr R1
  source 1..27: mol_type = other DNA
caccagtttcttacgcatcggtttctc

SEQ ID NO: 49 - DNA, 18 bp, synthetic construct
  misc_feature 1..18: note = Spegt1-tr F2
  source 1..18: mol_type = other DNA
cgatgcgtaagaaactgg

SEQ ID NO: 50 - DNA, 19 bp, synthetic construct
  misc_feature 1..19: note = Spegt1-tr R2
  source 1..19: mol_type = other DNA
aggcggtgtacatattgtc

SEQ ID NO: 51 - DNA, 19 bp, synthetic construct
  misc_feature 1..19: note = Spegt1-tr F3
  source 1..19: mol_type = other DNA
agccaccggctttcagcag

SEQ ID NO: 52 - DNA, 22 bp, synthetic construct
  misc_feature 1..22: note = Spegt1-tr R3
  source 1..22: mol_type = other DNA
caccagacgtgcaccaatccag

SEQ ID NO: 53 - DNA, 18 bp, synthetic construct
  misc_feature 1..18: note = Spegt1-tr F4
  source 1..18: mol_type = other DNA
ggattggtgcacgtctgg

SEQ ID NO: 54 - DNA, 17 bp, synthetic construct
  misc_feature 1..17: note = Spegt1-tr R4
  source 1..17: mol_type = other DNA
gctgctgaaagccggtg

SEQ ID NO: 55 - DNA, 21 bp, synthetic construct
  misc_feature 1..21: note = Spegt2 F1
  source 1..21: mol_type = other DNA
agatataccatgggcagcagc

SEQ ID NO: 56 - DNA, 25 bp, synthetic construct
  misc_feature 1..25: note = Spegt2 R1
  source 1..25: mol_type = other DNA
acagatcttcatcgatttcaacacc

SEQ ID NO: 57 - DNA, 25 bp, synthetic construct
  misc_feature 1..25: note = Spegt2 F2
  source 1..25: mol_type = other DNA
tgaaatcgatgaagatctgtttctg

SEQ ID NO: 58 - DNA, 19 bp, synthetic construct
  misc_feature 1..19: note = Spegt2 R2
  source 1..19: mol_type = other DNA
ctgctgcccatggtatatc

SEQ ID NO: 59 - DNA, 28 bp, synthetic construct
  misc_feature 1..28: note = Spegt2 F3
  source 1..28: mol_type = other DNA
ggtgttgaaatcgatgaagatctgtttc

SEQ ID NO: 60 - DNA, 23 bp, synthetic construct
  misc_feature 1..23: note = Spegt2 R3
  source 1..23: mol_type = other DNA
ctgctggattttttcttcgccac

SEQ ID NO: 61 - DNA, 20 bp, synthetic construct
  misc_feature 1..20: note = Spegt2 F4
  source 1..20: mol_type = other DNA
gcgaagaaaaaatccagcag

SEQ ID NO: 62 - DNA, 23 bp, synthetic construct
  misc_feature 1..23: note = Spegt2 R4
  source 1..23: mol_type = other DNA
tcttcatcgatttcaacaccaac